European Patent Application EP 4 201 958 A1, published June 28, 2023. Title: ANTI-CTLA-4 ANTIBODY AND USE THEREOF. Applicant: Suzhou Junmeng Biosciences Co., Ltd. The sequence listing filed with the application follows.

SEQUENCE LISTING (71 sequences)

SEQ ID NO: 1 - protein, 6 aa, Artificial sequence
  Synthetic polypeptide
SGYYWN

SEQ ID NO: 2 - protein, 16 aa, Artificial sequence
  Synthetic polypeptide
YIGYDGSNYYNPSLKN

SEQ ID NO: 3 - protein, 9 aa, Artificial sequence
  Synthetic polypeptide
NYYSGYFDF

SEQ ID NO: 4 - protein, 11 aa, Artificial sequence
  Synthetic polypeptide
KASQIVGSYVA

SEQ ID NO: 5 - protein, 7 aa, Artificial sequence
  Synthetic polypeptide
STSYRHS

SEQ ID NO: 6 - protein, 8 aa, Artificial sequence
  Synthetic polypeptide
QQHHLPLT

SEQ ID NO: 7 - protein, 5 aa, Artificial sequence
  Synthetic polypeptide
DYYMS

SEQ ID NO: 8 - protein, 19 aa, Artificial sequence
  Synthetic polypeptide
FIRNKANGFTAEYSASVKG

SEQ ID NO: 9 - protein, 13 aa, Artificial sequence
  Synthetic polypeptide
DSLAYPHYYAMDY

SEQ ID NO: 10 - protein, 10 aa, Artificial sequence
  Synthetic polypeptide
SASSSVSYMY

SEQ ID NO: 11 - protein, 7 aa, Artificial sequence
  Synthetic polypeptide
LTSNLAS

SEQ ID NO: 12 - protein, 9 aa, Artificial sequence
  Synthetic polypeptide
QQWSSNSFT

SEQ ID NO: 13 - protein, 5 aa, Artificial sequence
  Synthetic polypeptide
DTYMH

SEQ ID NO: 14 - protein, 17 aa, Artificial sequence
  Synthetic polypeptide
RIDPANGNTKSDPKFQG

SEQ ID NO: 15 - protein, 9 aa, Artificial sequence
  Synthetic polypeptide
SMTTDPFTY

SEQ ID NO: 16 - protein, 11 aa, Artificial sequence
  Synthetic polypeptide
KASQNVGTYVA

SEQ ID NO: 17 - protein, 7 aa, Artificial sequence
  Synthetic polypeptide
STSYRYS

SEQ ID NO: 18 - protein, 9 aa, Artificial sequence
  Synthetic polypeptide
HQYDTYPLT

SEQ ID NO: 19 - protein, 6 aa, Artificial sequence
  Synthetic polypeptide
SGYYWN

SEQ ID NO: 20 - protein, 16 aa, Artificial sequence
  Synthetic polypeptide
YIGYDGSNNYNPSLKN

SEQ ID NO: 21 - protein, 9 aa, Artificial sequence
  Synthetic polypeptide
DYYSGYFDS

SEQ ID NO: 22 - protein, 5 aa, Artificial sequence
  Synthetic polypeptide
DYYMK

SEQ ID NO: 23 - protein, 17 aa, Artificial sequence
  Synthetic polypeptide
HINPNNGDTFYNQKFTG

SEQ ID NO: 24 - protein, 11 aa, Artificial sequence
  Synthetic polypeptide
GGDGRGTWFAY

SEQ ID NO: 25 - protein, 15 aa, Artificial sequence
  Synthetic polypeptide
RASESVDSYGISFMN

SEQ ID NO: 26 - protein, 7 aa, Artificial sequence
  Synthetic polypeptide
AASNQGS

SEQ ID NO: 27 - protein, 9 aa, Artificial sequence
  Synthetic polypeptide
QQSKEVPPT

SEQ ID NO: 28 - protein, 118 aa, Artificial sequence
  Synthetic polypeptide
DVQLQESGQGLVKPSQSLSLTCSVTGYSITSGYYWNWIRQFPGNKLEWLGYIGYDGSNYYNPSLKNRISITRDTSKNQFFLKLNSVTSEDTATYFCARNYYSGYFDFWGQGTTLTVSS

SEQ ID NO: 29 - protein, 106 aa, Artificial sequence
  Synthetic polypeptide
DIVMTQSQKFMSTSVGDRVSVTCKASQIVGSYVAWYQQKLGQSPKALIYSTSYRHSGVPDRFTGSGSGTDFTLTISNVQSEDLAEYFCQQHHLPLTFGAGTKLEIK

SEQ ID NO: 30 - protein, 124 aa, Artificial sequence
  Synthetic polypeptide
EVKLVESGGGLVQPGGSLRLSCATSGFTFTDYYMSWVRQPPGKALEWLGFIRNKANGFTAEYSASVKGRFTISRDNSQSILYLQMNTLRAEDSATYYCARDSLAYPHYYAMDYWGQGTSVTVSS

SEQ ID NO: 31 - protein, 106 aa, Artificial sequence
  Synthetic polypeptide
QIVLTQSPALMSASPGEKVTMTCSASSSVSYMYWYQQKPRSSPKPWIYLTSNLASGVPVRFSGSGSGTSYSLTISSMEAEDAATYYCQQWSSNSFTFGSGTKLEIK

SEQ ID NO: 32 - protein, 118 aa, Artificial sequence
  Synthetic polypeptide
EVQLQQSGAELVKSGASVKLSCTGSGFNIKDTYMHWVKQRPEEGLEWIGRIDPANGNTKSDPKFQGKATITADTSSNTAYLQLSSLTSVDTAVYYCARSMTTDPFTYWGQGTLVTVSS

SEQ ID NO: 33 - protein, 107 aa, Artificial sequence
  Synthetic polypeptide
DIVMTQSQKFMSTSVGDSVSVTCKASQNVGTYVAWYQQKPGQSPKPLIYSTSYRYSGVPDRFTGSGSGTDFTLTISNVQSEDLAEYFCHQYDTYPLTFGAGTKLELK

SEQ ID NO: 34 - protein, 118 aa, Artificial sequence
  Synthetic polypeptide
DVQLQESGPGLVKPSQSLSLTCSVTAYSITSGYYWNWIRQFPGNKLEWMGYIGYDGSNNYNPSLKNRISITRDTSKNQFFLKLNSVTTEDTATYYCARDYYSGYFDSWGQGTTLTVSS

SEQ ID NO: 35 - protein, 120 aa, Artificial sequence
  Synthetic polypeptide
EVQLQQSGPELVKPGASVKMSCKASGYTFTDYYMKWMKQSHGKSLEWIGHINPNNGDTFYNQKFTGKATLTVDKSSSTASMHLNSLTSEDSAVYYCARGGDGRGTWFAYWGQGTLVTVSS

SEQ ID NO: 36 - protein, 111 aa, Artificial sequence
  Synthetic polypeptide
DIVLTQSPASLAEFLGQRATISCRASESVDSYGISFMNWFQQKPGQPPKLLIYAASNQGSGVPARFSGSGSGTDFSLNIHPMEEDDTAMYFCQQSKEVPPTFGGGTKLEIK

SEQ ID NO: 37 - protein, 16 aa, Artificial sequence
  Synthetic polypeptide
YIGYDGSNYYNPSLKS

SEQ ID NO: 38 - protein, 9 aa, Artificial sequence
  Synthetic polypeptide
NYYSGYFDS

SEQ ID NO: 39 - protein, 16 aa, Artificial sequence
  Synthetic polypeptide
YIGYDGSNNYNPSLKS

SEQ ID NO: 40 - protein, 11 aa, Artificial sequence
  Synthetic polypeptide
RASQNVGTYVA

SEQ ID NO: 41 - protein, 11 aa, Artificial sequence
  Synthetic polypeptide
QASQNVGTYVA

SEQ ID NO: 42 - protein, 118 aa, Artificial sequence
  Synthetic polypeptide
QVQLQESGPGLVKPSQTLSLTCTVSGYSISSGYYWNWIRQHPGKGLEWIGYIGYDGSNYYNPSLKSRVTISRDTSKNQFSLKLSSVTAADTAVYFCARNYYSGYFDFWGQGTTLTVSS

SEQ ID NO: 43 - protein, 118 aa, Artificial sequence
  Synthetic polypeptide
QVQLQESGPGLVKPSQTLSLTCTVSGYSITSGYYWNWIRQHPGKGLEWIGYIGYDGSNYYNPSLKSRVTISRDTSKNQFSLKLSSVTAADTAVYFCARNYYSGYFDFWGQGTTLTVSS

SEQ ID NO: 44 - protein, 118 aa, Artificial sequence
  Synthetic polypeptide
QVQLQESGPGLVKPSETLSLTCTVTGYSITSGYYWNWIRQPAGKGLEWIGYIGYDGSNYYNPSLKSRVTISRDTSKNQFSLKLSSVTAADTAVYFCARNYYSGYFDFWGQGTTLTVSS

SEQ ID NO: 45 - protein, 118 aa, Artificial sequence
  Synthetic polypeptide
QVQLQESGPGLVKPSQTLSLTCAVSGYSITSGYYWNWIRQHPGKGLEWIGYIGYDGSNYYNPSLKSRVTISRDTSKNQFSLKLSSVTAADTAVYFCARNYYSGYFDFWGQGTTLTVSS

SEQ ID NO: 46 - protein, 118 aa, Artificial sequence
  Synthetic polypeptide
QVQLQESGPGLVKPSQTLSLTCAVSGYSISSGYYWNWIRQPPGKGLEWIGYIGYDGSNYYNPSLKSRVTMSVDTSKNQFSLKLSSVTAVDTAVYYCARNYYSGYFDSWGQGTTVTVSS

SEQ ID NO: 47 - protein, 118 aa, Artificial sequence
  Synthetic polypeptide
QVQLQESGPGLVKPSQTLSLTCAVSGYSISSGYYWNWIRQFPGKGLEWMGYIGYDGSNYYNPSLKNRVTMSVDTSKNQFSLKLSSVTAVDTAVYYCARNYYSGYFDSWGQGTTVTVSS

SEQ ID NO: 48 - protein, 118 aa, Artificial sequence
  Synthetic polypeptide
QVQLQESGPGLVKPSQTLSLTCAVSGYSISSGYYWNWIRQPPGKGLEWIGYIGYDGSNYYNPSLKSRITISRDTSKNQFSLKLSSVTAVDTAVYYCARNYYSGYFDSWGQGTTVTVSS

SEQ ID NO: 49 - protein, 118 aa, Artificial sequence
  Synthetic polypeptide
QVQLQESGPGLVKPSQTLSLTCTVSGYSITSGYYWNWIRQHPGKGLEWIGYIGYDGSNNYNPSLKSRVTISRDTSKNQFSLKLSSVTAADTAVYYCARDYYSGYFDSWGQGTTLTVSS

SEQ ID NO: 50 - protein, 118 aa, Artificial sequence
  Synthetic polypeptide
QVQLQESGPGLVKPSQTLSLTCTVSAYSITSGYYWNWIRQHPGKGLEWIGYIGYDGSNNYNPSLKSRVTISRDTSKNQFSLKLSSVTAADTAVYYCARDYYSGYFDSWGQGTTLTVSS

SEQ ID NO: 51 - protein, 118 aa, Artificial sequence
  Synthetic polypeptide
QVQLQESGPGLVKPSETLSLTCTVSGYSITSGYYWNWIRQPPGKGLEWIGYIGYDGSNNYNPSLKSRVTISRDTSKNQFSLKLSSVTAADTAVYYCARDYYSGYFDSWGQGTTLTVSS

SEQ ID NO: 52 - protein, 118 aa, Artificial sequence
  Synthetic polypeptide
QVQLQESGPGLVKPSQTLSLTCAVSAYSITSGYYWNWIRQHPGKGLEWIGYIGYDGSNNYNPSLKSRVTISRDTSKNQFSLKLSSVTAADTAVYYCARDYYSGYFDSWGQGTTLTVSS

SEQ ID NO: 53 - protein, 118 aa, Artificial sequence
  Synthetic polypeptide
QVQLQESGPGLVKPSQTLSLTCAVSGYSITSGYYWNWIRQPPGKGLEWIGYIGYDGSNNYNPSLKNRVTMSVDTSKNQFSLKLSSVTAVDTAVYYCARDYYSGYFDSWGQGTTVTVSS

SEQ ID NO: 54 - protein, 107 aa, Artificial sequence
  Synthetic polypeptide
DIVMTQSPDSLAVSLGERATINCKASQNVGTYVAWYQQKPGQPPKPLIYSTSYRYSGVPDRFSGSGSGTDFTLTISSLQAEDVAVYFCHQYDTYPLTFGAGTKLELK

SEQ ID NO: 55 - protein, 107 aa, Artificial sequence
  Synthetic polypeptide
DIQMTQSPSSLSASVGDRVTITCRASQNVGTYVAWYQQKPGKVPKPLIYSTSYRYSGVPSRFSGSGSGTDFTLTISSLQPEDVATYFCHQYDTYPLTFGAGTKLELK

SEQ ID NO: 56 - protein, 107 aa, Artificial sequence
  Synthetic polypeptide
DIQMTQSPSSLSASVGDRVTITCRASQNVGTYVAWYQQKPGKAPKPLIYSTSYRYSGVPSRFSGSGSGTDFTLTISSLQPEDFATYFCHQYDTYPLTFGAGTKLELK

SEQ ID NO: 57 - protein, 107 aa, Artificial sequence
  Synthetic polypeptide
DIQMTQSPSFLSASVGDRVTITCRASQNVGTYVAWYQQKPGKAPKPLIYSTSYRYSGVPSRFSGSGSGTEFTLTISSLQPEDFATYFCHQYDTYPLTFGAGTKLELK

SEQ ID NO: 58 - protein, 107 aa, Artificial sequence
  Synthetic polypeptide
DIQMTQSPSSLSASVGDRVTITCQASQNVGTYVAWYQQKPGKAPKPLIYSTSYRYSGVPSRFSGSGSGTDFTFTISSLQPEDIATYFCHQYDTYPLTFGAGTKLELK

SEQ ID NO: 59 - protein, 107 aa, Artificial sequence
  Synthetic polypeptide
DIVMTQSPDSLAVSLGERATINCKASQNVGTYVAWYQQKPGQPPKLLIYSTSYRYSGVPDRFSGSGSGTDFTLTISSLQAEDVAVYYCHQYDTYPLTFGQGTKLEIK

SEQ ID NO: 60 - protein, 107 aa, Artificial sequence
  Synthetic polypeptide
EIVMTQSPATLSVSPGERATLSCRASQNVGTYVAWYQQKPGQAPRPLIYSTSYRYSGIPARFSGSGSGTEFTLTISSLQSEDFAVYYCHQYDTYPLTFGQGTKLEIK

SEQ ID NO: 61 - protein, 107 aa, Artificial sequence
  Synthetic polypeptide
DIVMTQSPDSLAVSLGERATINCKASQNVGTYVAWYQQKPGQPPKPLIYSTSYRYSGVPDRFSGSGSGTDFTLTISSLQAEDVAVYFCHQYDTYPLTFGQGTKLEIK

SEQ ID NO: 62 - protein, 107 aa, Artificial sequence
  Synthetic polypeptide
EIVMTQSPATLSVSPGERATLSCKASQNVGTYVAWYQQKPGQAPRPLIYSTSYRYSGIPARFSGSGSGTEFTLTISSLQSEDFAVYFCHQYDTYPLTFGQGTKLEIK

SEQ ID NO: 63 - protein, 448 aa, Artificial sequence
  Synthetic polypeptide
QVQLQESGPGLVKPSQTLSLTCTVSAYSITSGYYWNWIRQHPGKGLEWIGYIGYDGSNNYNPSLKSRVTISRDTSKNQFSLKLSSVTAADTAVYYCARDYYSGYFDSWGQGTTLTVSSASTKGPSVFPLAPSSKSTSGGTAALGCLVKDYFPEPVTVSWNSGALTSGVHTFPAVLQSSGLYSLSSVVTVPSSSLGTQTYICNVNHKPSNTKVDKKVEPKSCDKTHTCPPCPAPELLGGPSVFLFPPKPKDTLMISRTPEVTCVVVDVSHEDPEVKFNWYVDGVEVHNAKTKPREEQYNSTYRVVSVLTVLHQDWLNGKEYKCKVSNKALPAPIEKTISKAKGQPREPQVYTLPPSRDELTKNQVSLTCLVKGFYPSDIAVEWESNGQPENNYKTTPPVLDSDGSFFLYSKLTVDKSRWQQGNVFSCSVMHEALHNHYTQKSLSLSPGK

SEQ ID NO: 64 - protein, 214 aa, Artificial sequence
  Synthetic polypeptide
DIQMTQSPSSLSASVGDRVTITCRASQNVGTYVAWYQQKPGKVPKPLIYSTSYRYSGVPSRFSGSGSGTDFTLTISSLQPEDVATYFCHQYDTYPLTFGAGTKLELKRTVAAPSVFIFPPSDEQLKSGTASVVCLLNNFYPREAKVQWKVDNALQSGNSQESVTEQDSKDSTYSLSSTLTLSKADYEKHKVYACEVTHQGLSSPVTKSFNRGEC

SEQ ID NO: 65 - protein, 448 aa, Artificial sequence; identical to SEQ ID NO: 63
  Synthetic polypeptide

SEQ ID NO: 66 - protein, 214 aa, Artificial sequence
  Synthetic polypeptide
DIQMTQSPSSLSASVGDRVTITCRASQNVGTYVAWYQQKPGKAPKPLIYSTSYRYSGVPSRFSGSGSGTDFTLTISSLQPEDFATYFCHQYDTYPLTFGAGTKLELKRTVAAPSVFIFPPSDEQLKSGTASVVCLLNNFYPREAKVQWKVDNALQSGNSQESVTEQDSKDSTYSLSSTLTLSKADYEKHKVYACEVTHQGLSSPVTKSFNRGEC

SEQ ID NO: 67 - protein, 448 aa, Artificial sequence
  Synthetic polypeptide
QVQLQESGPGLVKPSQTLSLTCAVSGYSISSGYYWNWIRQPPGKGLEWIGYIGYDGSNYYNPSLKSRVTMSVDTSKNQFSLKLSSVTAVDTAVYYCARNYYSGYFDSWGQGTTVTVSSASTKGPSVFPLAPSSKSTSGGTAALGCLVKDYFPEPVTVSWNSGALTSGVHTFPAVLQSSGLYSLSSVVTVPSSSLGTQTYICNVNHKPSNTKVDKKVEPKSCDKTHTCPPCPAPELLGGPSVFLFPPKPKDTLMISRTPEVTCVVVDVSHEDPEVKFNWYVDGVEVHNAKTKPREEQYNSTYRVVSVLTVLHQDWLNGKEYKCKVSNKALPAPIEKTISKAKGQPREPQVYTLPPSRDELTKNQVSLTCLVKGFYPSDIAVEWESNGQPENNYKTTPPVLDSDGSFFLYSKLTVDKSRWQQGNVFSCSVMHEALHNHYTQKSLSLSPGK

SEQ ID NO: 68 - protein, 214 aa, Artificial sequence
  Synthetic polypeptide
EIVMTQSPATLSVSPGERATLSCRASQNVGTYVAWYQQKPGQAPRPLIYSTSYRYSGIPARFSGSGSGTEFTLTISSLQSEDFAVYYCHQYDTYPLTFGQGTKLEIKRTVAAPSVFIFPPSDEQLKSGTASVVCLLNNFYPREAKVQWKVDNALQSGNSQESVTEQDSKDSTYSLSSTLTLSKADYEKHKVYACEVTHQGLSSPVTKSFNRGEC

SEQ ID NO: 69 - protein, 448 aa, Artificial sequence
  Synthetic polypeptide
QVQLQESGPGLVKPSQTLSLTCAVSGYSITSGYYWNWIRQPPGKGLEWIGYIGYDGSNNYNPSLKNRVTMSVDTSKNQFSLKLSSVTAVDTAVYYCARDYYSGYFDSWGQGTTVTVSSASTKGPSVFPLAPSSKSTSGGTAALGCLVKDYFPEPVTVSWNSGALTSGVHTFPAVLQSSGLYSLSSVVTVPSSSLGTQTYICNVNHKPSNTKVDKKVEPKSCDKTHTCPPCPAPELLGGPSVFLFPPKPKDTLMISRTPEVTCVVVDVSHEDPEVKFNWYVDGVEVHNAKTKPREEQYNSTYRVVSVLTVLHQDWLNGKEYKCKVSNKALPAPIEKTISKAKGQPREPQVYTLPPSRDELTKNQVSLTCLVKGFYPSDIAVEWESNGQPENNYKTTPPVLDSDGSFFLYSKLTVDKSRWQQGNVFSCSVMHEALHNHYTQKSLSLSPGK

SEQ ID NO: 70 - protein, 214 aa, Artificial sequence; identical to SEQ ID NO: 68
  Synthetic polypeptide

SEQ ID NO: 71 - protein, 223 aa, Homo sapiens
  Human CTLA-4 protein
MACLGFQRHKAQLNLATRTWPCTLLFFLLFIPVFCKAMHVAQPAVVLASSRGIASFVCEYASPGKATEVRVTVLRQADSQVTEVCAATYMMGNELTFLDDSICTGTSSGNQVNLTIQGLRAMDTGLYICKVELMYPPPYYLGIGNGTQIYVIDPEPCPDSDFLLWILAAVSSGLFFYSFLLTAVSLSKMLKKRSPLTTGVYVKMPPTEPECEKQFQPYFIPIN